European Patent Application EP 4 803 614 A1, published September 9, 2026. Title: 一种表达多特异性抗原结合蛋白的细胞及其应用. Applicant: 苏州沙砾生物科技有限公司. Application WO. The sequence listing filed with the application follows.

SEQUENCE LISTING (60 sequences)

SEQ ID NO: 1 - protein, 35 aa, synthetic construct
MDAMKRGLCCVLLLCGAVFVSPSQEIHARFRRGAR

SEQ ID NO: 2 - protein, 20 aa, synthetic construct
GGGGSGGGGSGGGGSGGGGS

SEQ ID NO: 3 - protein, 8 aa, synthetic construct
DYKDDDDK

SEQ ID NO: 4 - protein, 8 aa, synthetic construct
HHHHHHHH

SEQ ID NO: 5 - protein, 27 aa, synthetic construct
RAKRSGSGATNFSLLKQAGDVEENPGP

SEQ ID NO: 6 - protein, 162 aa, synthetic construct
MNPAISVALLLSVLQVSRGQKVTSLTACLVNQNLRLDCRHENNTKDNSIQHEFSLTREKRKHVLSGTLGIPEHTYRSRVTLSNQPYIKVLTLANFTTKDEGDYFCELRVSGANPMSSNKSISVYRDKLVKCGGISLLVQNTSWMLLLLLSLSLLQALDFISL

SEQ ID NO: 7 - protein, 750 aa, synthetic construct
MDAMKRGLCCVLLLCGAVFVSPSQEIHARFRRGARQVQLVQSGAEVKKPGASVKVSCKASGYTFTSHWMHWVRQAPGQGLEWIGEFNPSNGRTNYNEKFKSKATMTVDTSTNTAYMELSSLRSEDTAVYYCASRDYDYDGRYFDYWGQGTLVTVSSGGGGSGGGGSGGGGSGGGGSDIQMTQSPSSLSASVGDRVTITCSASSSVTYMYWYQQKPGKAPKLLIYDTSNLASGVPSRFSGSGSGTDYTFTISSLQPEDIATYYCQQWSSHIFTFGQGTKVEIKGGGGSEVQLVESGGGLVQPKGSLKLSCAASGFTFNTYAMNWVRQAPGKGLEWVARIRSKYNNYATYYADSVKDRFTISRDDSQSLLYLQMNNLKTEDTAMYYCVRHGNFGNSYVSWFAYWGQGTLVTVSAGGGGSGGGGSGGGGSGGGGSQAVVTQESALTTSPGETVTLTCRSSTGAVTTSNYANWVQEKPDHLFTGLIGGTNKRAPGVPARFSGSLIGDKAALTITGAQTEDEAIYFCALWYSNLWVFGGGTKLTVLGSDYKDDDDKLEHHHHHHHHRAKRSGSGATNFSLLKQAGDVEENPGPMNPAISVALLLSVLQVSRGQKVTSLTACLVNQNLRLDCRHENNTKDNSIQHEFSLTREKRKHVLSGTLGIPEHTYRSRVTLSNQPYIKVLTLANFTTKDEGDYFCELRVSGANPMSSNKSISVYRDKLVKCGGISLLVQNTSWMLLLLLSLSLLQALDFISL

SEQ ID NO: 8 - protein, 749 aa, synthetic construct
MDAMKRGLCCVLLLCGAVFVSPSQEIHARFRRGARQVQLKQSGPGLVQPSQSLSITCTVSGFSLTNYGVHWVRQSPGKGLEWLGVIWSGGNTDYNTPFTSRLSINKDNSKSQVFFKMNSLQSNDTAIYYCARALTYYDYEFAYWGQGTLVTVSAGGGGSGGGGSGGGGSGGGGSDILLTQSPVILSVSPGERVSFSCRASQSIGTNIHWYQQRTNGSPRLLIKYASESISGIPSRFSGSGSGTDFTLSINSVESEDIADYYCQQNNNWPTTFGAGTKLELKGGGGSEVQLVESGGGLVQPKGSLKLSCAASGFTFNTYAMNWVRQAPGKGLEWVARIRSKYNNYATYYADSVKDRFTISRDDSQSLLYLQMNNLKTEDTAMYYCVRHGNFGNSYVSWFAYWGQGTLVTVSAGGGGSGGGGSGGGGSGGGGSQAVVTQESALTTSPGETVTLTCRSSTGAVTTSNYANWVQEKPDHLFTGLIGGTNKRAPGVPARFSGSLIGDKAALTITGAQTEDEAIYFCALWYSNLWVFGGGTKLTVLGSDYKDDDDKLEHHHHHHHHRAKRSGSGATNFSLLKQAGDVEENPGPMNPAISVALLLSVLQVSRGQKVTSLTACLVNQNLRLDCRHENNTKDNSIQHEFSLTREKRKHVLSGTLGIPEHTYRSRVTLSNQPYIKVLTLANFTTKDEGDYFCELRVSGANPMSSNKSISVYRDKLVKCGGISLLVQNTSWMLLLLLSLSLLQALDFISL

SEQ ID NO: 9 - protein, 759 aa, synthetic construct
MDAMKRGLCCVLLLCGAVFVSPSQEIHARFRRGARQVQLVQSGAEVKKPGASVKVSCKTSRYTFTEYTIHWVRQAPGQRLEWIGGINPNNGIPNYNQKFKGRVTITVDTSASTAYMELSSLRSEDTAVYYCARRRIAYGYDEGHAMDYWGQGTLVTVSSGGGGSGGGGSGGGGSGGGGSDIVMTQSPDSLAVSLGERATINCKSSQSLLYSRNQKNYLAWYQQKGQPPKLLIFWASTRESGVPDRFSGSGFGTDFTLTISSLQAEDVAVYYCQQYFSYPLTFGQGTKVEIKGGGGSEVQLVESGGGLVQPKGSLKLSCAASGFTFNTYAMNWVRQAPGKGLEWVARIRSKYNNYATYYADSVKDRFTISRDDSQSLLYLQMNNLKTEDTAMYYCVRHGNFGNSYVSWFAYWGQGTLVTVSAGGGGSGGGGSGGGGSGGGGSQAVVTQESALTTSPGETVTLTCRSSTGAVTTSNYANWVQEKPDHLFTGLIGGTNKRAPGVPARFSGSLIGDKAALTITGAQTEDEAIYFCALWYSNLWVFGGGTKLTVLGSDYKDDDDKLEHHHHHHHHRAKRSGSGATNFSLLKQAGDVEENPGPMNPAISVALLLSVLQVSRGQKVTSLTACLVNQNLRLDCRHENNTKDNSIQHEFSLTREKRKHVLSGTLGIPEHTYRSRVTLSNQPYIKVLTLANFTTKDEGDYFCELRVSGANPMSSNKSISVYRDKLVKCGGISLLVQNTSWMLLLLLSLSLLQALDFISL

SEQ ID NO: 10 - protein, 754 aa, synthetic construct
MDAMKRGLCCVLLLCGAVFVSPSQEIHARFRRGARQVQLKQSGAELVKPGASVKLSCKTSGYTFTENIIHWVKQRSGQGLEWIGWFHPGSGSIKYNEKKDKATLTADKSSSTVYMELSRLTSEDSAVYFCARHGGTGRGAMDYWGQGTSVTVSSGGGGSGGGGSGGGGSGGGGSDILMTQSPASSVVSLSGQRATISCRASKSVSTSAYSYMHWYQQKPGQPPKLLIYLASNLESGVPPRFSGSGSGTDFTLNIHPVEEEDAATYYCQHSRELPYTFGGGTKLEIKGGGGSEVQLVESGGGLVQPKGSLKLSCAASGFTFNTYAMNWVRQAPGKGLEWVARIRSKYNNYATYYADSVKDRFTISRDDSQSLLYLQMNNLKTEDTAMYYCVRHGNFGNSYVSWFAYWGQGTLVTVSAGGGGSGGGGSGGGGSGGGGSQAVVTQESALTTSPGETVTLTCRSSTGAVTTSNYANWVQEKPDHLFTGLIGGTNKRAPGVPARFSGSLIGDKAALTITGAQTEDEAIYFCALWYSNLWVFGGGTKLTVLGSDYKDDDDKLEHHHHHHHHRAKRSGSGATNFSLLKQAGDVEENPGPMNPAISVALLLSVLQVSRGQKVTSLTACLVNQNLRLDCRHENNTKDNSIQHEFSLTREKRKHVLSGTLGIPEHTYRSRVTLSNQPYIKVLTLANFTTKDEGDYFCELRVSGANPMSSNKSISVYRDKLVKCGGISLLVQNTSWMLLLLLSLSLLQALDFISL

SEQ ID NO: 11 - protein, 5 aa, synthetic construct
TYAMN

SEQ ID NO: 12 - protein, 19 aa, synthetic construct
RIRSKYNNYATYYADSVKD

SEQ ID NO: 13 - protein, 14 aa, synthetic construct
HGNFGNSYVSWFAY

SEQ ID NO: 14 - protein, 14 aa, synthetic construct
RSSTGAVTTSNYAN

SEQ ID NO: 15 - protein, 7 aa, synthetic construct
GTNKRAP

SEQ ID NO: 16 - protein, 9 aa, synthetic construct
ALWYSNLWV

SEQ ID NO: 17 - protein, 125 aa, synthetic construct
EVQLVESGGGLVQPKGSLKLSCAASGFTFNTYAMNWVRQAPGKGLEWVARIRSKYNNYATYYADSVKDRFTISRDDSQSLLYLQMNNLKTEDTAMYYCVRHGNFGNSYVSWFAYWGQGTLVTVSA

SEQ ID NO: 18 - protein, 109 aa, synthetic construct
QAVVTQESALTTSPGETVTLTCRSSTGAVTTSNYANWVQEKPDHLFTGLIGGTNKRAPGVPARFSGSLIGDKAALTITGAQTEDEAIYFCALWYSNLWVFGGGTKLTVL

SEQ ID NO: 19 - protein, 254 aa, synthetic construct
EVQLVESGGGLVQPKGSLKLSCAASGFTFNTYAMNWVRQAPGKGLEWVARIRSKYNNYATYYADSVKDRFTISRDDSQSLLYLQMNNLKTEDTAMYYCVRHGNFGNSYVSWFAYWGQGTLVTVSAGGGGSGGGGSGGGGSGGGGSQAVVTQESALTTSPGETVTLTCRSSTGAVTTSNYANWVQEKPDHLFTGLIGGTNKRAPGVPARFSGSLIGDKAALTITGAQTEDEAIYFCALWYSNLWVFGGGTKLTVL

SEQ ID NO: 20 - protein, 5 aa, synthetic construct
GGGGS

SEQ ID NO: 21 - protein, 5 aa, synthetic construct
SHWMH

SEQ ID NO: 22 - protein, 17 aa, synthetic construct
EFNPSNGRTNYNEKFKS

SEQ ID NO: 23 - protein, 12 aa, synthetic construct
RDYDYDGRYFDY

SEQ ID NO: 24 - protein, 10 aa, synthetic construct
SASSSVTYMY

SEQ ID NO: 25 - protein, 7 aa, synthetic construct
DTSNLAS

SEQ ID NO: 26 - protein, 9 aa, synthetic construct
QQWSSHIFT

SEQ ID NO: 27 - protein, 121 aa, synthetic construct [sequence omitted]

SEQ ID NO: 28 - protein, 106 aa, synthetic construct [sequence omitted]

SEQ ID NO: 29 - protein, 247 aa, synthetic construct
QVQLVQSGAEVKKPGASVKVSCKASGYTFTSHWMHWVRQAPGQGLEWIGEFNPSNGRTNYNEKFKSKATMTVDTSTNTAYMELSSLRSEDTAVYYCASRDYDYDGRYFDYWGQGTLVTVSSGGGGSGGGGSGGGGSGGGGSDIQMTQSPSSLSASVGDRVTITCSASSSVTYMYWYQQKPGKAPKLLIYDTSNLASGVPSRFSGSGSGTDYTFTISSLQPEDIATYYCQQWSSHIFTFGQGTKVEIK

SEQ ID NO: 30 - protein, 506 aa, synthetic construct
QVQLVQSGAEVKKPGASVKVSCKASGYTFTSHWMHWVRQAPGQGLEWIGEFNPSNGRTNYNEKFKSKATMTVDTSTNTAYMELSSLRSEDTAVYYCASRDYDYDGRYFDYWGQGTLVTVSSGGGGSGGGGSGGGGSGGGGSDIQMTQSPSSLSASVGDRVTITCSASSSVTYMYWYQQKPGKAPKLLIYDTSNLASGVPSRFSGSGSGTDYTFTISSLQPEDIATYYCQQWSSHIFTFGQGTKVEIKGGGGSEVQLVESGGGLVQPKGSLKLSCAASGFTFNTYAMNWVRQAPGKGLEWVARIRSKYNNYATYYADSVKDRFTISRDDSQSLLYLQMNNLKTEDTAMYYCVRHGNFGNSYVSWFAYWGQGTLVTVSAGGGGSGGGGSGGGGSGGGGSQAVVTQESALTTSPGETVTLTCRSSTGAVTTSNYANWVQEKPDHLFTGLIGGTNKRAPGVPARFSGSLIGDKAALTITGAQTEDEAIYFCALWYSNLWVFGGGTKLTVL

SEQ ID NO: 31 - protein, 5 aa, synthetic construct
NYGVH

SEQ ID NO: 32 - protein, 16 aa, synthetic construct
VIWSGGNTDYNTPFTS

SEQ ID NO: 33 - protein, 11 aa, synthetic construct
ALTYYDYEFAY

SEQ ID NO: 34 - protein, 11 aa, synthetic construct
RASQSIGTNIH

SEQ ID NO: 35 - protein, 7 aa, synthetic construct
YASESIS

SEQ ID NO: 36 - protein, 9 aa, synthetic construct
QQNNNWPTT

SEQ ID NO: 37 - protein, 119 aa, synthetic construct
QVQLKQSGPGLVQPSQSLSITCTVSGFSLTNYGVHWVRQSPGKGLEWLGVIWSGGNTDYNTPFTSRLSINKDNSKSQVFFKMNSLQSNDTAIYYCARALTYYDYEFAYWGQGTLVTVSA

SEQ ID NO: 38 - protein, 107 aa, synthetic construct
DILLTQSPVILSVSPGERVSFSCRASQSIGTNIHWYQQRTNGSPRLLIKYASESISGIPSRFSGSGSGTDFTLSINSVESEDIADYYCQQNNNWPTTFGAGTKLELK

SEQ ID NO: 39 - protein, 246 aa, synthetic construct
QVQLKQSGPGLVQPSQSLSITCTVSGFSLTNYGVHWVRQSPGKGLEWLGVIWSGGNTDYNTPFTSRLSINKDNSKSQVFFKMNSLQSNDTAIYYCARALTYYDYEFAYWGQGTLVTVSAGGGGSGGGGSGGGGSGGGGSDILLTQSPVILSVSPGERVSFSCRASQSIGTNIHWYQQRTNGSPRLLIKYASESISGIPSRFSGSGSGTDFTLSINSVESEDIADYYCQQNNNWPTTFGAGTKLELK

SEQ ID NO: 40 - protein, 505 aa, synthetic construct
QVQLKQSGPGLVQPSQSLSITCTVSGFSLTNYGVHWVRQSPGKGLEWLGVIWSGGNTDYNTPFTSRLSINKDNSKSQVFFKMNSLQSNDTAIYYCARALTYYDYEFAYWGQGTLVTVSAGGGGSGGGGSGGGGSGGGGSDILLTQSPVILSVSPGERVSFSCRASQSIGTNIHWYQQRTNGSPRLLIKYASESISGIPSRFSGSGSGTDFTLSINSVESEDIADYYCQQNNNWPTTFGAGTKLELKGGGGSEVQLVESGGGLVQPKGSLKLSCAASGFTFNTYAMNWVRQAPGKGLEWVARIRSKYNNYATYYADSVKDRFTISRDDSQSLLYLQMNNLKTEDTAMYYCVRHGNFGNSYVSWFAYWGQGTLVTVSAGGGGSGGGGSGGGGSGGGGSQAVVTQESALTTSPGETVTLTCRSSTGAVTTSNYANWVQEKPDHLFTGLIGGTNKRAPGVPARFSGSLIGDKAALTITGAQTEDEAIYFCALWYSNLWVFGGGTKLTVL

SEQ ID NO: 41 - protein, 5 aa, synthetic construct
EYTIH

SEQ ID NO: 42 - protein, 17 aa, synthetic construct
GINPNNGIPNYNQKFKG

SEQ ID NO: 43 - protein, 15 aa, synthetic construct
RRIAYGYDEGHAMDY

SEQ ID NO: 44 - protein, 17 aa, synthetic construct
KSSQSLLYSRNQKNYLA

SEQ ID NO: 45 - protein, 7 aa, synthetic construct
WASTRES

SEQ ID NO: 46 - protein, 9 aa, synthetic construct
QQYFSYPLT

SEQ ID NO: 47 - protein, 124 aa, synthetic construct
QVQLVQSGAEVKKPGASVKVSCKTSRYTFTEYTIHWVRQAPGQRLEWIGGINPNNGIPNYNQKFKGRVTITVDTSASTAYMELSSLRSEDTAVYYCARRRIAYGYDEGHAMDYWGQGTLVTVSS

SEQ ID NO: 48 - protein, 112 aa, synthetic construct
DIVMTQSPDSLAVSLGERATINCKSSQSLLYSRNQKNYLAWYQQKGQPPKLLIFWASTRESGVPDRFSGSGFGTDFTLTISSLQAEDVAVYYCQQYFSYPLTFGQGTKVEIK

SEQ ID NO: 49 - protein, 256 aa, synthetic construct
QVQLVQSGAEVKKPGASVKVSCKTSRYTFTEYTIHWVRQAPGQRLEWIGGINPNNGIPNYNQKFKGRVTITVDTSASTAYMELSSLRSEDTAVYYCARRRIAYGYDEGHAMDYWGQGTLVTVSSGGGGSGGGGSGGGGSGGGGSDIVMTQSPDSLAVSLGERATINCKSSQSLLYSRNQKNYLAWYQQKGQPPKLLIFWASTRESGVPDRFSGSGFGTDFTLTISSLQAEDVAVYYCQQYFSYPLTFGQGTKVEIK

SEQ ID NO: 50 - protein, 515 aa, synthetic construct
QVQLVQSGAEVKKPGASVKVSCKTSRYTFTEYTIHWVRQAPGQRLEWIGGINPNNGIPNYNQKFKGRVTITVDTSASTAYMELSSLRSEDTAVYYCARRRIAYGYDEGHAMDYWGQGTLVTVSSGGGGSGGGGSGGGGSGGGGSDIVMTQSPDSLAVSLGERATINCKSSQSLLYSRNQKNYLAWYQQKGQPPKLLIFWASTRESGVPDRFSGSGFGTDFTLTISSLQAEDVAVYYCQQYFSYPLTFGQGTKVEIKGGGGSEVQLVESGGGLVQPKGSLKLSCAASGFTFNTYAMNWVRQAPGKGLEWVARIRSKYNNYATYYADSVKDRFTISRDDSQSLLYLQMNNLKTEDTAMYYCVRHGNFGNSYVSWFAYWGQGTLVTVSAGGGGSGGGGSGGGGSGGGGSQAVVTQESALTTSPGETVTLTCRSSTGAVTTSNYANWVQEKPDHLFTGLIGGTNKRAPGVPARFSGSLIGDKAALTITGAQTEDEAIYFCALWYSNLWVFGGGTKLTVL

SEQ ID NO: 51 - protein, 5 aa, synthetic construct
ENIIH

SEQ ID NO: 52 - protein, 16 aa, synthetic construct
WFHPGSGSIKYNEKKD

SEQ ID NO: 53 - protein, 11 aa, synthetic construct
HGGTGRGAMDY

SEQ ID NO: 54 - protein, 15 aa, synthetic construct
RASKSVSTSAYSYMH

SEQ ID NO: 55 - protein, 7 aa, synthetic construct
LASNLES

SEQ ID NO: 56 - protein, 9 aa, synthetic construct
QHSRELPYT

SEQ ID NO: 57 - protein, 119 aa, synthetic construct
QVQLKQSGAELVKPGASVKLSCKTSGYTFTENIIHWVKQRSGQGLEWIGWFHPGSGSIKYNEKKDKATLTADKSSSTVYMELSRLTSEDSAVYFCARHGGTGRGAMDYWGQGTSVTVSS

SEQ ID NO: 58 - protein, 112 aa, synthetic construct
DILMTQSPASSVVSLSGQRATISCRASKSVSTSAYSYMHWYQQKPGQPPKLLIYLASNLESGVPPRFSGSGSGTDFTLNIHPVEEEDAATYYCQHSRELPYTFGGGTKLEIK

SEQ ID NO: 59 - protein, 251 aa, synthetic construct
QVQLKQSGAELVKPGASVKLSCKTSGYTFTENIIHWVKQRSGQGLEWIGWFHPGSGSIKYNEKKDKATLTADKSSSTVYMELSRLTSEDSAVYFCARHGGTGRGAMDYWGQGTSVTVSSGGGGSGGGGSGGGGSGGGGSDILMTQSPASSVVSLSGQRATISCRASKSVSTSAYSYMHWYQQKPGQPPKLLIYLASNLESGVPPRFSGSGSGTDFTLNIHPVEEEDAATYYCQHSRELPYTFGGGTKLEIK

SEQ ID NO: 60 - protein, 510 aa, synthetic construct
QVQLKQSGAELVKPGASVKLSCKTSGYTFTENIIHWVKQRSGQGLEWIGWFHPGSGSIKYNEKKDKATLTADKSSSTVYMELSRLTSEDSAVYFCARHGGTGRGAMDYWGQGTSVTVSSGGGGSGGGGSGGGGSGGGGSDILMTQSPASSVVSLSGQRATISCRASKSVSTSAYSYMHWYQQKPGQPPKLLIYLASNLESGVPPRFSGSGSGTDFTLNIHPVEEEDAATYYCQHSRELPYTFGGGTKLEIKGGGGSEVQLVESGGGLVQPKGSLKLSCAASGFTFNTYAMNWVRQAPGKGLEWVARIRSKYNNYATYYADSVKDRFTISRDDSQSLLYLQMNNLKTEDTAMYYCVRHGNFGNSYVSWFAYWGQGTLVTVSAGGGGSGGGGSGGGGSGGGGSQAVVTQESALTTSPGETVTLTCRSSTGAVTTSNYANWVQEKPDHLFTGLIGGTNKRAPGVPARFSGSLIGDKAALTITGAQTEDEAIYFCALWYSNLWVFGGGTKLTVL